European Patent Specification EP 3 705 572 B1, published November 12, 2025. Title: Novel inosine-5'-monophosphate dehydrogenase and method for producing 5'-inosine monophosphate using the same. Applicant: CJ CheilJedang Corporation. The sequence listing filed with the application follows.

SEQUENCE LISTING (26 sequences)

SEQ ID NO: 1 - DNA, 1521 bp, Unknown
  guaB NT
atgaccgaaaatcgtgtttctaccggtggagatgacccaaataaggttgcattgcatggcttgacgtttgatgacgtgctgctgctacctgccgaatccaatgttgttccgtcggaagtagacacttcggcgcagttcacccgcaatactcgtttaggtattcctttggcatcggctgcgatggacacggttactgaggcgcgcatggctattgccatggcacgccagggtggcattggtgtcttgcaccgcaacttgtcctcgcaagagcaggcggagcaggtcgaaatcgtcaagcgctctgagtccggcatggtcaccgaccctgtgaccgcgaatccagacatgactatccaggaagttgatgacctgtgtgcacgcttccgcatctctggtcttcctgtggtcaacgaagacggcaccttgttgggcatttgcaccaaccgcgatatgcgctttgagcgcgactattcccgcaaggtttctgacatcatgaccgctatgccgctggttgtggcaaaagaaggcgtcagcaaggaagaagccctggatctgctgtcgacgaacaaggtagaaaagctacctatcgttgataaaaacaacaagctggtcggtctgattaccgttaaagactttgttaagaccgaacagttcccgaattcctccaaggatgcttcgggccgcttgctagtagcagcaggtattggtaccggcgaggagtcttatgagcgtgcaggcttgcttgtcgatgccggcgtggacgttctcattgtcgactccgcacacgcgcacaataaccgcgtgctggaaatggtctcgcgcgtcaagaatgacttcggctccaagattgatgttgtcggcggcaacctggcaacacgctcggcagcaaaggcgatgattgaggctggcgcagacgccatcaaggtgggtattggtcctggttctatctgcaccacccgtgtggttgctggtgttggtgcaccacagattaccgcgatcatggaagcagctaccgtggcttctgctgcgggcgtgcctttgattgcagacggcggcatgcagtactccggtgacgttgctaaggctttggctgctggcgcggactcggtcatgctgggctcgatgttcgcaggcaccctggaggctcctggtgacatcgtgattgtcggcggcaagcagtacaagcgctaccgcggcatgggttcgatgggcgctatgcaaggccgtggcctctccggcgagaagcgttcttactccaaggaccgctacttccaggcagatgtgcgcagcgaagataagctggttccagaaggcgtggaaggcaaggttccttaccgcggcgaaattggtcagattacccaccagattgtgggcggtttgcgcgcggcaatgggctacactggctccgctactattgaagagctgaagaccaagcagttcgtgcgtattaccactgctggcttggctgagtcgcacccgcaccacctgcagcaaactgtagaagctccgaactaccgttaa

SEQ ID NO: 2 - protein, 506 aa, Unknown
  guaB AA
MTENRVSTGGDDPNKVALHGLTFDDVLLLPAESNVVPSEVDTSAQFTRNTRLGIPLASAAMDTVTEARMAIAMARQGGIGVLHRNLSSQEQAEQVEIVKRSESGMVTDPVTANPDMTIQEVDDLCARFRISGLPVVNEDGTLLGICTNRDMRFERDYSRKVSDIMTAMPLVVAKEGVSKEEALDLLSTNKVEKLPIVDKNNKLVGLITVKDFVKTEQFPNSSKDASGRLLVAAGIGTGEESYERAGLLVDAGVDVLIVDSAHAHNNRVLEMVSRVKNDFGSKIDVVGGNLATRSAAKAMIEAGADAIKVGIGPGSICTTRVVAGVGAPQITAIMEAATVASAAGVPLIADGGMQYSGDVAKALAAGADSVMLGSMFAGTLEAPGDIVIVGGKQYKRYRGMGSMGAMQGRGLSGEKRSYSKDRYFQADVRSEDKLVPEGVEGKVPYRGEIGQITHQIVGGLRAAMGYTGSATIEELKTKQFVRITTAGLAESHPHHLQQTVEAPNYR

SEQ ID NO: 3 - DNA, 1521 bp, Unknown
  guaB NT(A377T)
atgaccgaaaatcgtgtttctaccggtggagatgacccaaataaggttgcattgcatggcttgacgtttgatgacgtgctgctgctacctgccgaatccaatgttgttccgtcggaagtagacacttcggcgcagttcacccgcaatactcgtttaggtattcctttggcatcggctgcgatggacacggttactgaggcgcgcatggctattgccatggcacgccagggtggcattggtgtcttgcaccgcaacttgtcctcgcaagagcaggcggagcaggtcgaaatcgtcaagcgctctgagtccggcatggtcaccgaccctgtgaccgcgaatccagacatgactatccaggaagttgatgacctgtgtgcacgcttccgcatctctggtcttcctgtggtcaacgaagacggcaccttgttgggcatttgcaccaaccgcgatatgcgctttgagcgcgactattcccgcaaggtttctgacatcatgaccgctatgccgctggttgtggcaaaagaaggcgtcagcaaggaagaagccctggatctgctgtcgacgaacaaggtagaaaagctacctatcgttgataaaaacaacaagctggtcggtctgattaccgttaaagactttgttaagaccgaacagttcccgaattcctccaaggatgcttcgggccgcttgctagtagcagcaggtattggtaccggcgaggagtcttatgagcgtgcaggcttgcttgtcgatgccggcgtggacgttctcattgtcgactccgcacacgcgcacaataaccgcgtgctggaaatggtctcgcgcgtcaagaatgacttcggctccaagattgatgttgtcggcggcaacctggcaacacgctcggcagcaaaggcgatgattgaggctggcgcagacgccatcaaggtgggtattggtcctggttctatctgcaccacccgtgtggttgctggtgttggtgcaccacagattaccgcgatcatggaagcagctaccgtggcttctgctgcgggcgtgcctttgattgcagacggcggcatgcagtactccggtgacgttgctaaggctttggctgctggcgcggactcggtcatgctgggctcgatgttcacaggcaccctggaggctcctggtgacatcgtgattgtcggcggcaagcagtacaagcgctaccgcggcatgggttcgatgggcgctatgcaaggccgtggcctctccggcgagaagcgttcttactccaaggaccgctacttccaggcagatgtgcgcagcgaagataagctggttccagaaggcgtggaaggcaaggttccttaccgcggcgaaattggtcagattacccaccagattgtgggcggtttgcgcgcggcaatgggctacactggctccgctactattgaagagctgaagaccaagcagttcgtgcgtattaccactgctggcttggctgagtcgcacccgcaccacctgcagcaaactgtagaagctccgaactaccgttaa

SEQ ID NO: 4 - DNA, 1521 bp, Unknown
  guaB NT(T499I)
atgaccgaaaatcgtgtttctaccggtggagatgacccaaataaggttgcattgcatggcttgacgtttgatgacgtgctgctgctacctgccgaatccaatgttgttccgtcggaagtagacacttcggcgcagttcacccgcaatactcgtttaggtattcctttggcatcggctgcgatggacacggttactgaggcgcgcatggctattgccatggcacgccagggtggcattggtgtcttgcaccgcaacttgtcctcgcaagagcaggcggagcaggtcgaaatcgtcaagcgctctgagtccggcatggtcaccgaccctgtgaccgcgaatccagacatgactatccaggaagttgatgacctgtgtgcacgcttccgcatctctggtcttcctgtggtcaacgaagacggcaccttgttgggcatttgcaccaaccgcgatatgcgctttgagcgcgactattcccgcaaggtttctgacatcatgaccgctatgccgctggttgtggcaaaagaaggcgtcagcaaggaagaagccctggatctgctgtcgacgaacaaggtagaaaagctacctatcgttgataaaaacaacaagctggtcggtctgattaccgttaaagactttgttaagaccgaacagttcccgaattcctccaaggatgcttcgggccgcttgctagtagcagcaggtattggtaccggcgaggagtcttatgagcgtgcaggcttgcttgtcgatgccggcgtggacgttctcattgtcgactccgcacacgcgcacaataaccgcgtgctggaaatggtctcgcgcgtcaagaatgacttcggctccaagattgatgttgtcggcggcaacctggcaacacgctcggcagcaaaggcgatgattgaggctggcgcagacgccatcaaggtgggtattggtcctggttctatctgcaccacccgtgtggttgctggtgttggtgcaccacagattaccgcgatcatggaagcagctaccgtggcttctgctgcgggcgtgcctttgattgcagacggcggcatgcagtactccggtgacgttgctaaggctttggctgctggcgcggactcggtcatgctgggctcgatgttcgcaggcaccctggaggctcctggtgacatcgtgattgtcggcggcaagcagtacaagcgctaccgcggcatgggttcgatgggcgctatgcaaggccgtggcctctccggcgagaagcgttcttactccaaggaccgctacttccaggcagatgtgcgcagcgaagataagctggttccagaaggcgtggaaggcaaggttccttaccgcggcgaaattggtcagattacccaccagattgtgggcggtttgcgcgcggcaatgggctacactggctccgctactattgaagagctgaagaccaagcagttcgtgcgtattaccactgctggcttggctgagtcgcacccgcaccacctgcagcaaattgtagaagctccgaactaccgttaa

SEQ ID NO: 5 - DNA, 1521 bp, Unknown
  guaB NT(A377T, T499I)
atgaccgaaaatcgtgtttctaccggtggagatgacccaaataaggttgcattgcatggcttgacgtttgatgacgtgctgctgctacctgccgaatccaatgttgttccgtcggaagtagacacttcggcgcagttcacccgcaatactcgtttaggtattcctttggcatcggctgcgatggacacggttactgaggcgcgcatggctattgccatggcacgccagggtggcattggtgtcttgcaccgcaacttgtcctcgcaagagcaggcggagcaggtcgaaatcgtcaagcgctctgagtccggcatggtcaccgaccctgtgaccgcgaatccagacatgactatccaggaagttgatgacctgtgtgcacgcttccgcatctctggtcttcctgtggtcaacgaagacggcaccttgttgggcatttgcaccaaccgcgatatgcgctttgagcgcgactattcccgcaaggtttctgacatcatgaccgctatgccgctggttgtggcaaaagaaggcgtcagcaaggaagaagccctggatctgctgtcgacgaacaaggtagaaaagctacctatcgttgataaaaacaacaagctggtcggtctgattaccgttaaagactttgttaagaccgaacagttcccgaattcctccaaggatgcttcgggccgcttgctagtagcagcaggtattggtaccggcgaggagtcttatgagcgtgcaggcttgcttgtcgatgccggcgtggacgttctcattgtcgactccgcacacgcgcacaataaccgcgtgctggaaatggtctcgcgcgtcaagaatgacttcggctccaagattgatgttgtcggcggcaacctggcaacacgctcggcagcaaaggcgatgattgaggctggcgcagacgccatcaaggtgggtattggtcctggttctatctgcaccacccgtgtggttgctggtgttggtgcaccacagattaccgcgatcatggaagcagctaccgtggcttctgctgcgggcgtgcctttgattgcagacggcggcatgcagtactccggtgacgttgctaaggctttggctgctggcgcggactcggtcatgctgggctcgatgttcacaggcaccctggaggctcctggtgacatcgtgattgtcggcggcaagcagtacaagcgctaccgcggcatgggttcgatgggcgctatgcaaggccgtggcctctccggcgagaagcgttcttactccaaggaccgctacttccaggcagatgtgcgcagcgaagataagctggttccagaaggcgtggaaggcaaggttccttaccgcggcgaaattggtcagattacccaccagattgtgggcggtttgcgcgcggcaatgggctacactggctccgctactattgaagagctgaagaccaagcagttcgtgcgtattaccactgctggcttggctgagtcgcacccgcaccacctgcagcaaattgtagaagctccgaactaccgttaa

SEQ ID NO: 6 - protein, 506 aa, Unknown
  GuaB(A377T)-AA
MTENRVSTGGDDPNKVALHGLTFDDVLLLPAESNVVPSEVDTSAQFTRNTRLGIPLASAAMDTVTEARMAIAMARQGGIGVLHRNLSSQEQAEQVEIVKRSESGMVTDPVTANPDMTIQEVDDLCARFRISGLPVVNEDGTLLGICTNRDMRFERDYSRKVSDIMTAMPLVVAKEGVSKEEALDLLSTNKVEKLPIVDKNNKLVGLITVKDFVKTEQFPNSSKDASGRLLVAAGIGTGEESYERAGLLVDAGVDVLIVDSAHAHNNRVLEMVSRVKNDFGSKIDVVGGNLATRSAAKAMIEAGADAIKVGIGPGSICTTRVVAGVGAPQITAIMEAATVASAAGVPLIADGGMQYSGDVAKALAAGADSVMLGSMFTGTLEAPGDIVIVGGKQYKRYRGMGSMGAMQGRGLSGEKRSYSKDRYFQADVRSEDKLVPEGVEGKVPYRGEIGQITHQIVGGLRAAMGYTGSATIEELKTKQFVRITTAGLAESHPHHLQQTVEAPNYR

SEQ ID NO: 7 - protein, 506 aa, Unknown
  GuaB(T499I)-AA
MTENRVSTGGDDPNKVALHGLTFDDVLLLPAESNVVPSEVDTSAQFTRNTRLGIPLASAAMDTVTEARMAIAMARQGGIGVLHRNLSSQEQAEQVEIVKRSESGMVTDPVTANPDMTIQEVDDLCARFRISGLPVVNEDGTLLGICTNRDMRFERDYSRKVSDIMTAMPLVVAKEGVSKEEALDLLSTNKVEKLPIVDKNNKLVGLITVKDFVKTEQFPNSSKDASGRLLVAAGIGTGEESYERAGLLVDAGVDVLIVDSAHAHNNRVLEMVSRVKNDFGSKIDVVGGNLATRSAAKAMIEAGADAIKVGIGPGSICTTRVVAGVGAPQITAIMEAATVASAAGVPLIADGGMQYSGDVAKALAAGADSVMLGSMFAGTLEAPGDIVIVGGKQYKRYRGMGSMGAMQGRGLSGEKRSYSKDRYFQADVRSEDKLVPEGVEGKVPYRGEIGQITHQIVGGLRAAMGYTGSATIEELKTKQFVRITTAGLAESHPHHLQQIVEAPNYR

SEQ ID NO: 8 - protein, 506 aa, Unknown
  GuaB(A377T,T499I)-AA
MTENRVSTGGDDPNKVALHGLTFDDVLLLPAESNVVPSEVDTSAQFTRNTRLGIPLASAAMDTVTEARMAIAMARQGGIGVLHRNLSSQEQAEQVEIVKRSESGMVTDPVTANPDMTIQEVDDLCARFRISGLPVVNEDGTLLGICTNRDMRFERDYSRKVSDIMTAMPLVVAKEGVSKEEALDLLSTNKVEKLPIVDKNNKLVGLITVKDFVKTEQFPNSSKDASGRLLVAAGIGTGEESYERAGLLVDAGVDVLIVDSAHAHNNRVLEMVSRVKNDFGSKIDVVGGNLATRSAAKAMIEAGADAIKVGIGPGSICTTRVVAGVGAPQITAIMEAATVASAAGVPLIADGGMQYSGDVAKALAAGADSVMLGSMFTGTLEAPGDIVIVGGKQYKRYRGMGSMGAMQGRGLSGEKRSYSKDRYFQADVRSEDKLVPEGVEGKVPYRGEIGQITHQIVGGLRAAMGYTGSATIEELKTKQFVRITTAGLAESHPHHLQQIVEAPNYR

SEQ ID NO: 9 - DNA, 29 bp, Artificial Sequence
  pDZ-purF(g1a)-1
gctctagaccactctaagacgcggccacc

SEQ ID NO: 10 - DNA, 37 bp, Artificial Sequence
  pDZ-purF(g1a)-2
aagtagtgttcaccatgacgctgattctactaagttt

SEQ ID NO: 11 - DNA, 38 bp, Artificial Sequence
  pDZ-purF(g1a)-3
agtagaatcagcgtcatggtgaacactactttccccag

SEQ ID NO: 12 - DNA, 29 bp, Artificial Sequence
  pDZ-purF(g1a)-4
gctctagactgtgcgcccacgatatccag

SEQ ID NO: 13 - DNA, 29 bp, Artificial Sequence
  pDZ-purA(a1t)-1
gctctagaggccacgatgcccggagcatc

SEQ ID NO: 14 - DNA, 37 bp, Artificial Sequence
  pDZ-purA(a1t)-2
taacgatagctgccaaggttattcacttcctagattt

SEQ ID NO: 15 - DNA, 37 bp, Artificial Sequence
  pDZ-purA(a1t)-3
aggaagtgaataaccttggcagctatcgttatcgtcg

SEQ ID NO: 16 - DNA, 29 bp, Artificial Sequence
  pDZ-purA(a1t)-4
gctctagaggtcacgaatgggtaggtgcc

SEQ ID NO: 17 - DNA, 21 bp, Artificial Sequence
  pCR-guaB-F
actgcattacacggatatgta

SEQ ID NO: 18 - DNA, 21 bp, Artificial Sequence
  pCR-guaB-R
cctcgtggcgtccccacaaac

SEQ ID NO: 19 - DNA, 21 bp, Artificial Sequence
  pTOPO-guaB-library-F
attgcatggcttgacgtttga

SEQ ID NO: 20 - DNA, 21 bp, Artificial Sequence
  pTOPT-guaB-library-R
atcaatgtgccactgcgtgct

SEQ ID NO: 21 - DNA, 21 bp, Artificial Sequence
  guaB seq F
aatgaaagatgccggatcatt

SEQ ID NO: 22 - DNA, 21 bp, Artificial Sequence
  guaB seq R
acgcccgaatcacgaacctga

SEQ ID NO: 23 - DNA, 75 bp, Artificial Sequence
  mage A337T
acaatcacgatgtcaccaggagcctccagggtgcctgtgaacatcgagcccagcatgaccgagtccgcgccagca

SEQ ID NO: 24 - DNA, 75 bp, Artificial Sequence
  mage T499I
tatttttaatccttaacggtagttcggagcttctacaatttgctgcaggtggtgcgggtgcgactcagccaagcc

SEQ ID NO: 25 - DNA, 29 bp, Artificial Sequence
  pDZ-guaB-F
gctctagagacatgactatccaggaagtt

SEQ ID NO: 26 - DNA, 29 bp, Artificial Sequence
  pDZ-guaB-R
gctctagacagtggtgtaatccaccacgc